European Patent Specification EP 3 655 431 B1, published May 21, 2025. Title: Anti- isoAsp7 amyloid β (Aβ) antibodies and uses thereof. Applicant: FRAUNHOFER-GESELLSCHAFT ZUR FÖRDERUNG DER ANGEWANDTEN FORSCHUNG E V. The sequence listing filed with the application follows.

SEQUENCE LISTING (68 sequences)

SEQ ID NO: 1 - protein, 42 aa, Artificial Sequence [sequence omitted]

SEQ ID NO: 2 - protein, 40 aa, Artificial Sequence
  Aβ 1-40
DAEFRHDSGYEVHHQKLVFFAEDVGSNKGAIIGLMVGGVV

SEQ ID NO: 3 - protein, 13 aa, Artificial Sequence
  isoD7-Aβ(1-12)Cys
  MOD_RES 7: L-IsoAsp
DAEFRHXSGYEVC

SEQ ID NO: 4 - protein, 16 aa, Artificial Sequence
  isoD7-Aβ(5-9)repCys
  MOD_RES 3: L-IsoAsp
  MOD_RES 8: L-IsoAsp
  MOD_RES 13: L-IsoAsp
RHXSGRHXSGRHXSGC

SEQ ID NO: 5 - protein, 18 aa, Artificial Sequence
  isoD7-Aβ(1-18)PEG-Biotin
  MOD_RES 7: L-IsoAsp
  MOD_RES 18: PEG-Biotin
DAEFRHXSGYEVHHQKLV

SEQ ID NO: 6 - protein, 18 aa, Artificial Sequence
  Aβ(1-18)PEG-Biotin
  MOD_RES 18: PEG-Biotin
DAEFRHDSGYEVHHQKLV

SEQ ID NO: 7 - protein, 17 aa, Artificial Sequence
  isod7-Aβ(1-17)
  MOD_RES 7: D-IsoAsp
DAEFRHXSGYEVHHQKL

SEQ ID NO: 8 - protein, 18 aa, Artificial Sequence
  Aβ(1-18)
DAEFRHDSGYEVHHQKLV

SEQ ID NO: 9 - protein, 17 aa, Artificial Sequence
  K11 LCDR1
KSSQSLLNSRNRKNYLA

SEQ ID NO: 10 - protein, 17 aa, Artificial Sequence
  K11 LCDR1 consensus
  VARIANT 9: S or R
  VARIANT 11: N or T
KSSQSLLNXRXRKNYLA

SEQ ID NO: 11 - protein, 7 aa, Artificial Sequence
  K11 LCDR2
WASTRDS

SEQ ID NO: 12 - protein, 7 aa, Artificial Sequence
  K11 LCDR2 consensus
  VARIANT 6: D or E
WASTRXS

SEQ ID NO: 13 - protein, 8 aa, Artificial Sequence
  K11 LCDR3
KQSYNLRT

SEQ ID NO: 14 - protein, 10 aa, Artificial Sequence
  K11 HCDR1
GFSLTSYGVH

SEQ ID NO: 15 - protein, 16 aa, Artificial Sequence
  K11 HCDR2
ALWASGNTDYSSTLMS

SEQ ID NO: 16 - protein, 16 aa, Artificial Sequence
  K11 HCDR2 consensus
  VARIANT 1: A or V
  VARIANT 7: N or R
  VARIANT 11: S or N
  VARIANT 13: T or A
XLWASGXTDYXSXLMS

SEQ ID NO: 17 - protein, 12 aa, Artificial Sequence
  K11 HCDR3
DRGILTGGYFDV

SEQ ID NO: 18 - protein, 12 aa, Artificial Sequence
  K11 HCDR3 consensus
  VARIANT 5: L, T or M
DRGIXTGGYFDV

SEQ ID NO: 19 - protein, 112 aa, Artificial Sequence
  K11 VL
DIVMSQSPTSLAVSAGEKVTMSCKSSQSLLNSRNRKNYLAWYQQKPGQSPKLLIYWASTRDSGVPDRFTGSGSGTDFTLTISSVQAEDLAVYYCKQSYNLRTFGGGTKLEIK

SEQ ID NO: 20 - protein, 120 aa, Artificial Sequence
  K11 VH
QVQLKESGPGLVAPSQSLSITCTVSGFSLTSYGVHWVRQPPGKGLEWLGALWASGNTDYSSALMSRLSISKDNSKSQVFLKMNSLQTDDTAMYYCARDRGIMTGGYFDVWGAGTTVTVSS

SEQ ID NO: 21 - protein, 219 aa, Artificial Sequence
  K11 LC
DIVMSQSPTSLAVSAGEKVTMSCKSSQSLLNSRNRKNYLAWYQQKPGQSPKLLIYWASTRDSGVPDRFTGSGSGTDFTLTISSVQAEDLAVYYCKQSYNLRTFGGGTKLEIKRADAAPTVSIFPPSSEQLTSGGASVVCFLNNFYPKDINVKWKIDGSERQNGVLNSWTDQDSKDSTYSMSSTLTLTKDEYERHNSYTCEATHKTSTSPIVKSFNRNEC

SEQ ID NO: 22 - protein, 444 aa, Artificial Sequence
  K11 HC
QVQLKESGPGLVAPSQSLSITCTVSGFSLTSYGVHWVRQPPGKGLEWLGALWASGNTDYSSTLMSRLSISKDNSKSQVFLKMNSLQTDDTAMYYCARDRGILTGGYFDVWGAGTTVTVSSAKTTPPSVYPLAPGSAAQTNSMVTLGCLVKGYFPEPVTVTWNSGSLSSGVHTFPAVLQSDLYTLSSSVTVPSSTWPSETVTCNVAHPASSTKVDKKIVPRDCGCKPCICTVPEVSSVFIFPPKPKDVLTITLTPKVTCVVVDISKDDPEVQFSWFVDDVEVHTAQTQPREEQFNSTFRSVSELPIMHQDWLNGKEFKCRVNSAAFPAPIEKTISKTKGRPKAPQVYTIPPPKEQMAKDKVSLTCMITDFFPEDITVEWQWNGQPAENYKNTQPIMDTDGSYFVYSKLNVQKSNWEAGNTFTCSVLHEGLHNHHTEKSLSHSPGK

SEQ ID NO: 23 - DNA, 336 bp, Artificial Sequence
  K11 VL DNA
gacattgtgatgtcacagtctccaacctccctggctgtgtcagcaggagagaaggtcaccatgagctgcaaatccagtcagagtctactcaacagtagaaaccgaaagaactacttggcttggtaccagcagaaaccagggcagtctcctaaactgctgatctactgggcatccactagggattctggggtccctgatcgcttcacaggcagtggatctgggacagatttcactctcaccatcagcagtgtgcaggctgaagacctggcagtttattactgcaagcaatcttataatcttcggacgttcggtggaggcaccaagctggaaatcaaa

SEQ ID NO: 24 - DNA, 360 bp, Artificial Sequence
  K11 VH DNA
caggtgcagctgaaggagtcaggacctggcctggtggcgccctcacagagcctgtccatcacttgcactgtctctggattttcattaaccagctatggtgtacactgggttcgccagcctccaggaaagggtctggagtggctgggagcactatgggctagtggaaacacagattatagttcgactctcatgtccagactgagcatcagcaaagacaactccaagagccaagttttcttaaaaatgaacagtctgcaaactgatgacacagccatgtattactgtgccagagatcgggggattctgacgggagggtacttcgatgtctggggcgcagggaccacggtcaccgtctcctca

SEQ ID NO: 25 - DNA, 657 bp, Artificial Sequence
  K11 LC DNA
gacattgtgatgtcacagtctccaacctccctggctgtgtcagcaggagagaaggtcaccatgagctgcaaatccagtcagagtctactcaacagtagaaaccgaaagaactacttggcttggtaccagcagaaaccagggcagtctcctaaactgctgatctactgggcatccactagggattctggggtccctgatcgcttcacaggcagtggatctgggacagatttcactctcaccatcagcagtgtgcaggctgaagacctggcagtttattactgcaagcaatcttataatcttcggacgttcggtggaggcaccaagctggaaatcaaacgggctgatgctgcaccaactgtatccatcttcccaccatccagtgagcagttaacatctggaggtgcctcagtcgtgtgcttcttgaacaacttctaccccaaagacatcaatgtcaagtggaagattgatggcagtgaacgacaaaatggcgtcctgaacagttggactgatcaggacagcaaagacagcacctacagcatgagcagcaccctcacgttgaccaaggacgagtatgaacgacataacagctatacctgtgaggccactcacaagacatcaacttcacccattgtcaagagcttcaacaggaatgagtgt

SEQ ID NO: 26 - DNA, 1332 bp, Artificial Sequence
  K11 HC DNA
caggtgcagctgaaggagtcaggacctggcctggtggcgccctcacagagcctgtccatcacttgcactgtctctggattttcattaaccagctatggtgtacactgggttcgccagcctccaggaaagggtctggagtggctgggagcactatgggctagtggaaacacagattatagttcgactctcatgtccagactgagcatcagcaaagacaactccaagagccaagttttcttaaaaatgaacagtctgcaaactgatgacacagccatgtattactgtgccagagatcgggggattctgacgggagggtacttcgatgtctggggcgcagggaccacggtcaccgtctcctcagccaaaacgacacccccatctgtctatccactggcccctggatctgctgcccaaactaactccatggtgaccctgggatgcctggtcaagggctatttccctgagccagtgacagtgacctggaactctggatccctgtccagcggtgtgcacaccttcccagctgtcctgcagtctgacctctacactctgagcagctcagtgactgtcccctccagccctcggcccagcgagaccgtcacctgcaacgttgcccacccggccagcagcaccaaggtggacaagaaaattgtgcccagggattgtggttgtaagccttgcatatgtacagtcccagaagtatcatctgtcttcatcttccccccaaagcccaaggatgtcctcaccattactctgactcctaaggtcacgtgtgttgtggtagacatcagcaaggatgatcccgaggtccagttcagctggtttgtagatgatgtggaggtgcacacagctcagacgcaaccccgggaggagcagttcaacagcactttccgctcagtcagtgaacttcccatcatgcaccaggactggctcaatggcaaggagttcaaatgcagggtcaacagtgcagctttccctgcccccatcgagaaaaccatatccaaaaccaaaggcagaccgaaggctccacaggtgtacaccattccacctcccaaggagcagatggccaaggataaagtcagtctgacctgcatgataacagacttcttccctgaagacataacagtggagtggcagtggaatgggcagccagcggagaactacaagaacactcagcccatcatgaacacgaatggctcttacttcgtctacagcaagctcaatgtgcagaagagcaactgggaggcaggaaatactttcacctgctctgtgttacatgagggcctgcacaaccaccatactgagaagagcctctcccactctcctggtaaa

SEQ ID NO: 27 - protein, 17 aa, Artificial Sequence
  K119 LCDR1
KSSQSLFNSRTRKNYVA

SEQ ID NO: 28 - protein, 17 aa, Artificial Sequence
  K119 LCDR1 consensus
  VARIANT 5: S or N
  VARIANT 7: F or L
  VARIANT 16: V or L
KSSQXLXNSRTRKNYXA

SEQ ID NO: 29 - protein, 7 aa, Artificial Sequence
  K119 LCDR2
WASTRES

SEQ ID NO: 30 - protein, 8 aa, Artificial Sequence
  K119 LCDR3
KQSYNLRA

SEQ ID NO: 31 - protein, 8 aa, Artificial Sequence
  K119 LCDR3 consensus
  VARIANT 1: K or M
  VARIANT 8: A or T
XQSYNLRX

SEQ ID NO: 32 - protein, 10 aa, Artificial Sequence
  K119 HCDR1
GFTFTDYYMS

SEQ ID NO: 33 - protein, 10 aa, Artificial Sequence
  K119 HCDR1 consensus
  VARIANT 5: T or S
  VARIANT 10: S or N
GFTFXDYYMX

SEQ ID NO: 34 - protein, 19 aa, Artificial Sequence
  K119 HCDR2
FIRNKANGYTTEYSASVKG

SEQ ID NO: 35 - protein, 8 aa, Artificial Sequence
  K119 HCDR3
DIPTIMDY

SEQ ID NO: 36 - protein, 112 aa, Artificial Sequence
  K119 VL
DIVMSQSPSSLAVSAGEKATMSCKSSQSLFNSRTRKNYVAWLQQKPGQSPKLLISWASTRESGVPDRFTGSGSGTDFALTITNVQAEDLAVYYCKQSYNLRAFGGGTKLEIT

SEQ ID NO: 37 - protein, 119 aa, Artificial Sequence
  K119 VH
EVKLVESGGGLVQPGGSLRLSCATSGFTFTDYYMSWVRQPPGKALEWLGFIRNKANGYTTEYSASVKGRFTISRDNSQSILYLQMNTLRTEDSATYYCTRDIPTIMDYWGQGTSVTVSS

SEQ ID NO: 38 - protein, 219 aa, Artificial Sequence
  K119 LC
DIVMSQSPSSLAVSAGEKATMSCKSSQSLFNSRTRKNYVAWLQQKPGQSPKLLISWASTRESGVPDRFTGSGSGTDFALTITNVQAEDLAVYYCKQSYNLRAFGGGTKLEITRADAAPTVSIFPPSSEQLTSGGASVVCFLNNFYPKDINVKWKIDGSERQNGVLNSWTDQDSKDSTYSMSSTLTLTKDEYERHNSYTCEATHKTSTSPIVKSFNRNEC

SEQ ID NO: 39 - protein, 449 aa, Artificial Sequence
  K119 HC
EVKLVESGGGLVQPGGSLRLSCATSGFTFTDYYMSWVRQPPGKALEWLGFIRNKANGYTTEYSASVKGRFTISRDNSQSILYLQMNTLRTEDSATYYCTRDIPTIMDYWGQGTSVTVSSAKTTAPSVYPLAPVCGDTTGSSVTLGCLVKGYFPEPVTLTWNSGSLSSGVHTFPAVLQSDLYTLSSSVTVTSSTWPSQSITCNVAHPASSTKVDKKIEPRGPTIKPCPPCKCPAPNLLGGPSVFIFPPKIKDVLMISLSPIVTCVVVDVSEDDPDVQISWFVNNVEVHTAQTQTHREDYNSTLRVVSALPIQHQDWMSGKEFKCKVNNKDLPAPIERTISKPKGSVRAPQVYVLPPPEEEMTKKQVTLTCMVTDFMPEDIYVEWTNNGKTELNYKNTEPVLDSDGSYFMYSKLRVEKKNWVERNSYSCSVVHEGLHNHHTTKSFSRTPGK

SEQ ID NO: 40 - DNA, 336 bp, Artificial Sequence
  K119 VL DNA
gacattgtgatgtcacagtctccatcctccctggctgtgtcagcaggagagaaggccactatgagctgcaaatccagtcagagtctgttcaacagtagaacccgaaagaactacgtggcttggctccagcagaaaccagggcagtctcctaaactactgatctcctgggcatccactagggaatctggggtccctgatcgcttcacaggcagtggatctgggacagatttcgctctcaccatcaccaatgtgcaggctgaagacctggcagtttattactgcaagcaatcttataatcttcgggcgttcggtggaggcaccaagctggaaatcaca

SEQ ID NO: 41 - DNA, 357 bp, Artificial Sequence
  K119 VH DNA
gaggtgaagctggtggagtctggaggaggcttggtacagcctgggggttctctgagactctcctgtgcaacttctgggttcaccttcactgattattatatgagctgggtccgccagcctccaggaaaggcacttgagtggttgggttttattagaaacaaagctaatggttatacaacagagtacagtgcatctgtgaagggtcggttcaccatctccagagataattcccaaagcatcctctatcttcaaatgaacaccctgagaactgaggacagtgccacttattactgtacaagagatatccccactatcatggactactggggtcaaggaacctcagtcaccgtctcctca

SEQ ID NO: 42 - DNA, 657 bp, Artificial Sequence
  K119 LC DNA
gacattgtgatgtcacagtctccatcctccctggctgtgtcagcaggagagaaggccactatgagctgcaaatccagtcagagtctgttcaacagtagaacccgaaagaactacgtggcttggctccagcagaaaccagggcagtctcctaaactactgatctcctgggcatccactagggaatctggggtccctgatcgcttcacaggcagtggatctgggacagatttcgctctcaccatcaccaatgtgcaggctgaagacctggcagtttattactgcaagcaatcttataatcttcgggcgttcggtggaggcaccaagctggaaatcacacgggctgatgctgcaccaactgtatccatcttcccaccatccagtgagcagttaacatctggaggtgcctcagtcgtgtgcttcttgaacaacttctaccccaaagacatcaatgtcaagtggaagattgatggcagtgaacgacaaaatggcgtcctgaacagttggactgatcaggacagcaaagacagcacctacagcatgagcagcaccctcacgttgaccaaggacgagtatgaacgacataacagctatacctgtgaggccactcacaagacatcaacttcacccattgtcaagagcttcaacaggaatgagtgt

SEQ ID NO: 43 - DNA, 1347 bp, Artificial Sequence
  K119 HC DNA
gaggtgaagctggtggagtctggaggaggcttggtacagcctgggggttctctgagactctcctgtgcaacttctgggttcaccttcactgattattatatgagctgggtccgccagcctccaggaaaggcacttgagtggttgggttttattagaaacaaagctaatggttatacaacagagtacagtgcatctgtgaagggtcggttcaccatctccagagataattcccaaagcatcctctatcttcaaatgaacaccctgagaactgaggacagtgccacttattactgtacaagagatatccccactatcatggactactggggtcaaggaacctcagtcaccgtctcctcagccaaaacaacagccccatcggtctatccactggcccctgtgtgtggagatacaactggctcctcggtgactctaggatgcctggtcaagggttatttccctgagccagtgaccttgacctggaactctggatccctgtccagtggtgtgcacaccttcccagctgtcctgcagtctgacctctacaccctcagcagctcagtgactgtaacctcgagcacctggcccagccagtccatcacctgcaatgtggcccacccggcaagcagcaccaaggtggacaagaaaattgagcccagagggcccacaatcaagccctgtcctccatgcaaatgcccagcacctaacctcttgggtggaccatccgtcttcatcttccctccaaagatcaaggatgtactcatgatctccctgagccccatagtcacatgtgtggtggtggatgtgagcgaggatgacccagatgtccagatcagctggtttgtgaacaacgtggaagtacacacagctcagacacaaacccatagagaggattacaacagtactctccgggtggtcagtgccctccccatccagcaccaggactggatgagtggcaaggagttcaaatgcaaggtcaacaacaaagacctcccagcgcccatcgagagaaccatctcaaaacccaaagggtcagtaagagctccacaggtatatgtcttgcctccaccagaagaagagatgactaagaaacaggtcactctgacctgcatggtcacagacttcatgcctgaagacatttacgtggagtggaccaacaacgggaaaacagagctaaactacaagaacactgaaccagtcctggactctgatggttcttacttcatgtacagcaagctgagagtggaaaagaagaactgggtggaaagaaatagctactcctgttcagtggtccacgagggtctgcacaatcaccacacgactaagagcttctcccggactccgggtaaa

SEQ ID NO: 44 - protein, 18 aa, Artificial Sequence
  isoD7-Aβ(1-18)
  MOD_RES 7: L-IsoAsp
DAEFRHXSGYEVHHQKLV

SEQ ID NO: 45 - protein, 40 aa, Artificial Sequence
  isoD7-Aβ(1-40)
  MOD_RES 7: L-IsoAsp
DAEFRHXSGYEVHHQKLVFFAEDVGSNKGAIIGLMVGGVV

SEQ ID NO: 46 - protein, 18 aa, Artificial Sequence
  isoD7-3nitroY10-Aβ(1-18)
  MOD_RES 7: L-IsoAsp
  MOD_RES 10: 3-Nitrotyrosine
DAEFRHXSGXEVHHQKLV

SEQ ID NO: 47 - protein, 16 aa, Artificial Sequence
  MOD_RES 1: L-pyroglutamate
  pE3-Aβ(3-18)
XFRHDSGYEVHHQKLV

SEQ ID NO: 48 - protein, 16 aa, Artificial Sequence
  MOD_RES 1: L-pyroglutamate
  pE3-isoD7-Aβ(3-18)
  MOD_RES 5: L-IsoAsp
XFRHXSGYEVHHQKLV

SEQ ID NO: 49 - protein, 18 aa, Artificial Sequence
  isoD7-phosphoSer8-Aβ(1-18)
  MOD_RES 7: L-IsoAsp
  MOD_RES 8: Phosphoserine
DAEFRHXXGYEVHHQKLV

SEQ ID NO: 50 - protein, 18 aa, Artificial Sequence
  Mouse isoD7-Aβ(1-18)
  MOD_RES 7: L-IsoAsp
DAEFGHXSGFEVRHQKLV

SEQ ID NO: 51 - protein, 30 aa, Artificial Sequence
  isoD7-Aβ(1-30)
  MOD_RES 7: L-IsoAsp
DAEFRHXSGYEVHHQKLVFFAEDVGSNKGA

SEQ ID NO: 52 - protein, 30 aa, Artificial Sequence
  Aβ(1-30)
DAEFRHDSGYEVHHQKLVFFAEDVGSNKGA

SEQ ID NO: 53 - protein, 112 aa, Artificial Sequence
  hVL11-IGKV4-1
DIVMTQSPDSLAVSLGERATINCKSSQSLLNSRNRKNYLAWYQQKPGQPPKLLIYWASTRDSGVPDRFSGSGSGTDFTLTISSLQAEDVAVYYCKQSYNLRTFGQGTKLEIK

SEQ ID NO: 54 - DNA, 336 bp, Artificial Sequence
  hVL11-IGKV4-1 DNA
gacatcgtgatgacacagagccccgattctctggccgtgtctctgggagagagagccaccatcaactgcaagagcagccagagcctgctgaacagccggaaccggaagaattacctggcctggtatcagcagaagcccggccagcctcctaagctgctgatctactgggccagcaccagagatagcggcgtgcccgatagattttctggctctggcagcggcaccgacttcaccctgacaatttctagcctgcaagccgaggacgtggccgtgtactactgcaagcagagctacaacctgcggacctttggccagggcaccaagctggaaatcaaa

SEQ ID NO: 55 - protein, 112 aa, Artificial Sequence
  hVL11-IGKV3-20*01
EIVLTQSPGTLSLSPGERATLSCKSSQSLLNSRNRKNYLAWYQQKPGQAPRLLIYWASTRDSGIPDRFSGSGSGTDYTLTISRLEPEDFAVYYCKQSYNLRTFGGGTKVEIK

SEQ ID NO: 56 - DNA, 336 bp, Artificial Sequence
  hVL11-IGKV3-20*01 DNA
gagatcgtgctgacacagagccccggaacactgtcactgtctccaggcgaaagagccacactgagctgcaagagcagccagagcctgctgaacagccggaaccggaagaattacctggcctggtatcagcagaagcccggacaggctcctcggctgctgatctattgggccagcacaagagacagcggcatccccgatagattttccggcagcggcagcggaaccgactacaccctgacaatcagcagactggaacccgaggacttcgccgtgtactactgcaagcagagctacaacctgcggacctttggcggaggcaccaaggtggaaatcaaa

SEQ ID NO: 57 - protein, 219 aa, Artificial Sequence
  hLC11-IGKV4-1 (kappa)
DIVMTQSPDSLAVSLGERATINCKSSQSLLNSRNRKNYLAWYQQKPGQPPKLLIYWASTRDSGVPDRFSGSGSGTDFTLTISSLQAEDVAVYYCKQSYNLRTFGQGTKLEIKRTVAAPSVFIFPPSDEQLKSGTASVVCLLNNFYPREAKVQWKVDNALQSGNSQESVTEQDSKDSTYSLSSTLTLSKADYEKHKVYACEVTHQGLSSPVTKSFNRGEC

SEQ ID NO: 58 - DNA, 657 bp, Artificial Sequence
  hLC11-IGKV4-1 (kappa) DNA
gacatcgtgatgacacagagccccgattctctggccgtgtctctgggagagagagccaccatcaactgcaagagcagccagagcctgctgaacagccggaaccggaagaattacctggcctggtatcagcagaagcccggccagcctcctaagctgctgatctactgggccagcaccagagatagcggcgtgcccgatagattttctggctctggcagcggcaccgacttcaccctgacaatttctagcctgcaagccgaggacgtggccgtgtactactgcaagcagagctacaacctgcggacctttggccagggcaccaagctggaaatcaaaaggaccgtggccgcaccctctgtgttcatcttcccccccagcgacgagcagctgaagagcggcactgcatctgtcgtgtgtctgctgaacaacttctacccaagggaggcgaaagtgcagtggaaggtagacaacgccttgcaatccggcaactcccaggagagcgtgaccgagcaggacagcaaagactcaacctacagcctgagcagtactttgaccctgtctaaggccgattacgagaagcacaaggtgtacgcctgcgaggtaacccaccagggactgagctctcccgtgaccaagagcttcaacaggggcgagtgc

SEQ ID NO: 59 - protein, 219 aa, Artificial Sequence
  hLC11-IGKV3-20*01 (kappa)
EIVLTQSPGTLSLSPGERATLSCKSSQSLLNSRNRKNYLAWYQQKPGQAPRLLIYWASTRDSGIPDRFSGSGSGTDYTLTISRLEPEDFAVYYCKQSYNLRTFGGGTKVEIKRTVAAPSVFIFPPSDEQLKSGTASVVCLLNNFYPREAKVQWKVDNALQSGNSQESVTEQDSKDSTYSLSSTLTLSKADYEKHKVYACEVTHQGLSSPVTKSFNRGEC

SEQ ID NO: 60 - DNA, 657 bp, Artificial Sequence
  hLC11-IGKV3-20*01 (kappa) DNA
gagatcgtgctgacacagagccccggaacactgtcactgtctccaggcgaaagagccacactgagctgcaagagcagccagagcctgctgaacagccggaaccggaagaattacctggcctggtatcagcagaagcccggacaggctcctcggctgctgatctattgggccagcacaagagacagcggcatccccgatagattttccggcagcggcagcggaaccgactacaccctgacaatcagcagactggaacccgaggacttcgccgtgtactactgcaagcagagctacaacctgcggacctttggcggaggcaccaaggtggaaatcaaaaggaccgtggccgcaccctctgtgttcatcttcccccccagcgacgagcagctgaagagcggcactgcatctgtcgtgtgtctgctgaacaacttctacccaagggaggcgaaagtgcagtggaaggtagacaacgccttgcaatccggcaactcccaggagagcgtgaccgagcaggacagcaaagactcaacctacagcctgagcagtactttgaccctgtctaaggccgattacgagaagcacaaggtgtacgcctgcgaggtaacccaccagggactgagctctcccgtgaccaagagcttcaacaggggcgagtgc

SEQ ID NO: 61 - protein, 120 aa, Artificial Sequence
  hVH11-IGHV4-4
QVQLQESGPGLVKPSGTLSLTCAVSGFSLTSYGVHWVRQPPGKGLEWLGALWASGNTDYSSTLMSRVTISVDKSKNQFSLRLSSVTAADTAVYYCARDRGILTGGYFDVWGKGTTVTVSS

SEQ ID NO: 62 - DNA, 360 bp, Artificial Sequence
  hVH11-IGHV4-4 DNA
caggttcagctgcaagaatctggccctggcctggtcaagcctagcggaacactgtctctgacctgtgccgtgtccggctttagcctgacaagctatggggtgcactgggtccgacagcctccaggcaaaggactggaatggctgggagcactgtgggcctctggcaacacagattacagcagcaccctgatgagcagagtgaccatcagcgtggacaagagcaagaaccagttcagcctgcggctgagcagcgtgacagctgctgatacagccgtgtactactgcgccagagacagaggcattctgaccggcggctacttcgatgtgtggggcaagggaaccaccgtgaccgttagttct

SEQ ID NO: 63 - protein, 120 aa, Artificial Sequence
  hVH11-IGHV4-59
QVQLQESGPGLVKPSETLSLTCTVSGFSLTSYGVHWIRQPPGKGLEWLGALWASGNTDYSSTLMSRVTISVDTSKNQFSLKLSSVTAADTAVYYCARDRGILTGGYFDLWGRGTLVTVSS

SEQ ID NO: 64 - DNA, 360 bp, Artificial Sequence
  hVH11-IGHV4-59 DNA
caggttcagctgcaagaatctggccctggcctggtcaagcctagcgagacactgagcctgacctgtaccgtgtccggctttagcctgacaagctacggggtgcactggatcagacagcctccaggcaaaggcctggaatggctgggagcactttgggcctctggcaacaccgattacagcagcaccctgatgagcagagtgaccatcagcgtggacaccagcaagaaccagttcagcctgaagctgagcagcgtgacagccgccgatacagccgtgtactactgcgccagagacagaggcattctgaccggcggctacttcgatctgtggggcagaggaacactggtcaccgtcagttct

SEQ ID NO: 65 - protein, 450 aa, Artificial Sequence
  hHC11-IGHV4-4 (IgG1)
QVQLQESGPGLVKPSGTLSLTCAVSGFSLTSYGVHWVRQPPGKGLEWLGALWASGNTDYSSTLMSRVTISVDKSKNQFSLRLSSVTAADTAVYYCARDRGILTGGYFDVWGKGTTVTVSSASTKGPSVFPLAPSSKSTSGGTAALGCLVKDYFPEPVTVSWNSGALTSGVHTFPAVLQSSGLYSLSSVVTVPSSSLGTQTYICNVNHKPSNTKVDKKVEPKSCDKTHTCPPCPAPELLGGPSVFLFPPKPKDTLMISRTPEVTCVVVDVSHEDPEVKFNWYVDGVEVHNAKTKPREEQYNSTYRVVSVLTVLHQDWLNGKEYKCKVSNKALPAPIEKTISKAKGQPREPQVYTLPPSRDELTKNQVSLTCLVKGFYPSDIAVEWESNGQPENNYKTTPPVLDSDGSFFLYSKLTVDKSRWQQGNVFSCSVMHEALHNHYTQKSLSLSPGK

SEQ ID NO: 66 - DNA, 1350 bp, Artificial Sequence
  hHC11-IGHV4-4 (IgG1) DNA
caggttcagctgcaagaatctggccctggcctggtcaagcctagcggaacactgtctctgacctgtgccgtgtccggctttagcctgacaagctatggggtgcactgggtccgacagcctccaggcaaaggactggaatggctgggagcactgtgggcctctggcaacacagattacagcagcaccctgatgagcagagtgaccatcagcgtggacaagagcaagaaccagttcagcctgcggctgagcagcgtgacagctgctgatacagccgtgtactactgcgccagagacagaggcattctgaccggcggctacttcgatgtgtggggcaagggaaccaccgtgaccgttagttctgccagcactaagggcccgagcgtgttccccctcgcccctagcagtaagagcaccagcggtggcacggcggcacttggctgcttggttaaggactacttcccagagcccgtgaccgtgtcctggaactctggggcacttaccagtggcgtgcacaccttccccgctgtactgcagagcagcggcttgtacagcttgtcttccgtcgtaacggtgcccagcagcagcttgggaacccagacctacatctgcaacgtaaaccacaagccatccaacaccaaggtagacaaaaaggtcgaacccaagtcctgcgacaagacccacacctgtccaccctgtcctgcacccgagctcctgggaggtcccagcgttttcctgttccctccaaagccaaaggataccctgatgatcagcaggacccccgaggtgacctgcgtggtggtggacgtgagccacgaagaccctgaggtcaagttcaactggtacgttgatggggtggaggtacacaatgccaagaccaaacctcgagaggagcaatacaacagcacctaccgagttgtgagcgtgcttaccgtgctgcaccaggactggctgaacggcaaggagtacaagtgcaaggtgagcaacaaggctctgccggctcccatcgagaagaccatcagcaaggccaagggccagcccagggagccacaggtttacacgttgcccccctcaagggacgagttgaccaagaaccaggtttccctcacgtgccttgtgaagggcttctaccccagcgacatcgccgtggaatgggagagcaacgggcagcccgagaacaactacaagacgaccccccctgttctggacagcgacggctctttcttcctgtattcaaagctcaccgtggacaaaagcaggtggcagcagggtaatgtgttctcctgcagcgtgatgcacgaggccctgcataaccactacacccaaaagagcttgagcctctcccccggtaag

SEQ ID NO: 67 - protein, 450 aa, Artificial Sequence
  hHC11-IGHV4-59 (IgG1)
QVQLQESGPGLVKPSETLSLTCTVSGFSLTSYGVHWIRQPPGKGLEWLGALWASGNTDYSSTLMSRVTISVDTSKNQFSLKLSSVTAADTAVYYCARDRGILTGGYFDLWGRGTLVTVSSASTKGPSVFPLAPSSKSTSGGTAALGCLVKDYFPEPVTVSWNSGALTSGVHTFPAVLQSSGLYSLSSVVTVPSSSLGTQTYICNVNHKPSNTKVDKKVEPKSCDKTHTCPPCPAPELLGGPSVFLFPPKPKDTLMISRTPEVTCVVVDVSHEDPEVKFNWYVDGVEVHNAKTKPREEQYNSTYRVVSVLTVLHQDWLNGKEYKCKVSNKALPAPIEKTISKAKGQPREPQVYTLPPSRDELTKNQVSLTCLVKGFYPSDIAVEWESNGQPENNYKTTPPVLDSDGSFFLYSKLTVDKSRWQQGNVFSCSVMHEALHNHYTQKSLSLSPGK

SEQ ID NO: 68 - DNA, 1350 bp, Artificial Sequence
  hHC11-IGHV4-59 (IgG1) DNA
caggttcagctgcaagaatctggccctggcctggtcaagcctagcgagacactgagcctgacctgtaccgtgtccggctttagcctgacaagctacggggtgcactggatcagacagcctccaggcaaaggcctggaatggctgggagcactttgggcctctggcaacaccgattacagcagcaccctgatgagcagagtgaccatcagcgtggacaccagcaagaaccagttcagcctgaagctgagcagcgtgacagccgccgatacagccgtgtactactgcgccagagacagaggcattctgaccggcggctacttcgatctgtggggcagaggaacactggtcaccgtcagttctgccagcactaagggcccgagcgtgttccccctcgcccctagcagtaagagcaccagcggtggcacggcggcacttggctgcttggttaaggactacttcccagagcccgtgaccgtgtcctggaactctggggcacttaccagtggcgtgcacaccttccccgctgtactgcagagcagcggcttgtacagcttgtcttccgtcgtaacggtgcccagcagcagcttgggaacccagacctacatctgcaacgtaaaccacaagccatccaacaccaaggtagacaaaaaggtcgaacccaagtcctgcgacaagacccacacctgtccaccctgtcctgcacccgagctcctgggaggtcccagcgttttcctgttccctccaaagccaaaggataccctgatgatcagcaggacccccgaggtgacctgcgtggtggtggacgtgagccacgaagaccctgaggtcaagttcaactggtacgttgatggggtggaggtacacaatgccaagaccaaacctcgagaggagcaatacaacagcacctaccgagttgtgagcgtgcttaccgtgctgcaccaggactggctgaacggcaaggagtacaagtgcaaggtgagcaacaaggctctgccggctcccatcgagaagaccatcagcaaggccaagggccagcccagggagccacaggtttacacgttgcccccctcaagggacgagttgaccaagaaccaggtttccctcacgtgccttgtgaagggcttctaccccagcgacatcgccgtggaatgggagagcaacgggcagcccgagaacaactacaagacgaccccccctgttctggacagcgacggctctttcttcctgtattcaaagctcaccgtggacaaaagcaggtggcagcagggtaatgtgttctcctgcagcgtgatgcacgaggccctgcataaccactacacccaaaagagcttgagcctctcccccggtaag